European Patent Application EP 4 201 960 A1, published June 28, 2023. Title: SINGLE VARIABLE DOMAIN AND ANTIGEN BINDING MOLECULE BINDING BCMA. Applicant: CHIA TAI TIANQING PHARMACEUTICAL GROUP CO., LTD. Application EP21857623.9. The sequence listing filed with the application follows.

SEQUENCE LISTING (36 sequences)

SEQ ID NO: 1 - DNA, 23 bp, Artificial Sequence
  Primer Sequence of Call001
gtcctggctgctcttctacaagg

SEQ ID NO: 2 - DNA, 23 bp, Artificial Sequence
  Primer Sequence of Call002
ggtacgtgctgttgaactgttcc

SEQ ID NO: 3 - DNA, 29 bp, Artificial Sequence
  Primer Sequence of V-Back
gatgtgcagctgcaggagtctggrggagg

SEQ ID NO: 4 - DNA, 34 bp, Artificial Sequence
  Primer Sequence of V-Fwd
ctagtgcggccgctgaggagacggtgacctgggt

SEQ ID NO: 5 - protein, 232 aa, Homo sapiens
EPKSCDKTHTCPPCPAPELLGGPSVFLFPPKPKDTLMISRTPEVTCVVVDVSHEDPEVKFNWYVDGVEVHNAKTKPREEQYNSTYRVVSVLTVLHQDWLNGKEYKCKVSNKALPAPIEKTISKAKGQPREPQVYTLPPSRDELTKNQVSLTCLVKGFYPSDIAVEWESNGQPENNYKTTPPVLDSDGSFFLYSKLTVDKSRWQQGNVFSCSVMHEALHNHYTQKSLSLSPGK

SEQ ID NO: 6 - protein, 183 aa, Macaca fascicularis
MLQMARQCSQNEYFDSLLHDCKPCQLRCSSTPPLTCQRYCNASMTNSVKGMNAILWTCLGLSLIISLAVFVLTFLLRKMSSEPLKDEFKNTGSGLLGMANIDLEKGRTGDEIVLPRGLEYTVEECTCEDCIKNKPKVDSDHCFPLPAMEEGATILVTTKTNDYCNSLSAALSVTEIEKSISAR

SEQ ID NO: 7 - protein, 5 aa, Camelus bactrianus
GWNKH

SEQ ID NO: 8 - protein, 16 aa, Camelus bactrianus
SIFRDGKTAYTDSVKG

SEQ ID NO: 9 - protein, 10 aa, Camelus bactrianus
DLPGSGLPAF

SEQ ID NO: 10 - protein, 5 aa, Camelus bactrianus
VACMA

SEQ ID NO: 11 - protein, 17 aa, Camelus bactrianus
TIVADFGTTNYAASVKG

SEQ ID NO: 12 - protein, 14 aa, Camelus bactrianus
TQRGGIDWCDEINY

SEQ ID NO: 13 - protein, 5 aa, Camelus bactrianus
SACMG

SEQ ID NO: 14 - protein, 17 aa, Camelus bactrianus
RIETGYGGTVYADSVKG

SEQ ID NO: 15 - protein, 17 aa, Camelus bactrianus
KRSWCTPTWWHELDYNY

SEQ ID NO: 16 - protein, 5 aa, Camelus bactrianus
GWNKH

SEQ ID NO: 17 - protein, 16 aa, Camelus bactrianus
SIFRDGKTAYTDSVKG

SEQ ID NO: 18 - protein, 10 aa, Camelus bactrianus
DLPGSGLPEF

SEQ ID NO: 19 - protein, 118 aa, Camelus bactrianus
QVQLVESGGGSVQAGGSLRLSCTASGYTFRGWNKHWYRQAPGKERELVSSIFRDGKTAYTDSVKGRFTISQDNADATVYLQMNSLKPEDTAMYYCKYDLPGSGLPAFWGQGTLVTVSS

SEQ ID NO: 20 - DNA, 354 bp, Camelus bactrianus
caggtgcagctggtggagtctgggggaggctcggtgcaggccggagggtctctgagactctcctgtacagcctctggatacaccttcaggggctggaacaagcactggtaccgccaggctccagggaaggagcgcgagttggtctcgagcatctttcgtgatgggaagacagcctatacagactccgtgaagggccgattcaccatctctcaagacaacgccgacgcaacggtgtatctgcaaatgaacagcctgaaacctgaggacacggccatgtattactgtaaatacgatctgcctggatctggtcttcctgcattctggggccaggggaccctggtcactgtctcatca

SEQ ID NO: 21 - protein, 123 aa, Camelus bactrianus
QVQLVESGGGSVQAGGSLRLSCAASGYSSNVACMAWYRQAPGKEREWVATIVADFGTTNYAASVKGRFTISQDNAKNTVYLQMNSLKPEDSAMYYCAATQRGGIDWCDEINYWGQGTLVTVSS

SEQ ID NO: 22 - DNA, 369 bp, Camelus bactrianus
caggtgcagctggtggagtctgggggaggctcggtgcaggctggagggtcgctgagactctcctgtgccgcctccggatacagcagtaatgtggcatgcatggcctggtaccgccaggctccagggaaggagcgcgagtgggtcgcaactattgttgctgatttcggtaccacaaactatgccgcctccgtgaagggccgattcaccatctcccaagacaacgccaagaacacggtgtatctgcaaatgaacagcctgaaacctgaggactctgccatgtactactgtgcggcaacccagagggggggtattgactggtgtgatgaaattaattactggggccaggggaccctggtcactgtctcatca

SEQ ID NO: 23 - protein, 126 aa, Camelus bactrianus
QVQLVESGGGSVQAGGSLRLSCAASGVTFNSACMGWFRQAPGKEREGVARIETGYGGTVYADSVKGRFTISRDNAKNTVYLQMNSLKPEDTAMYYCAAKRSWCTPTWWHELDYNYWGQGTQVTVSS

SEQ ID NO: 24 - DNA, 378 bp, Camelus bactrianus
caggtgcagctggtggagtctgggggaggctcggtgcaggctggagggtctctgagactctcctgtgcagcctctggagtcacttttaatagcgcatgtatgggttggttccgccaggctccagggaaggagcgcgagggggtcgcacgtattgaaactggttatggtggcactgtctatgccgactccgtgaagggacgattcaccatctcccgagacaacgccaagaacacggtgtatctgcaaatgaacagcctaaaacctgaggacactgccatgtactactgtgcggctaagagatcctggtgtactcctacgtggtggcacgaacttgactataactactggggacaggggacccaggtcactgtctcatca

SEQ ID NO: 25 - protein, 118 aa, Camelus bactrianus
EVQLVESGGGSVQAGGSLRLSCTASGYTFRGWNKHWYRQAPGKERELVSSIFRDGKTAYTDSVKGRFTISQDSADATVYLQMNSLKPEDTAMYYCKYDLPGSGLPEFWGQGTLVTVSS

SEQ ID NO: 26 - DNA, 354 bp, Camelus bactrianus
gaggtgcagctggtggagtctgggggaggctcggtgcaggccggagggtctctgagactctcctgtacagcctctggatacaccttcaggggctggaacaagcactggtaccgccaggctccagggaaggagcgcgagttggtctcgagtatctttcgtgatgggaagacagcctatacagactccgtgaagggccgattcaccatctctcaagacagcgccgacgcaacggtgtatctgcaaatgaacagcctgaaacctgaggacacggccatgtattactgtaaatacgatctgcctggatctggtcttcctgagttctggggccaggggaccctggtcactgtctcatca

SEQ ID NO: 27 - protein, 350 aa, Artificial Sequence
  the amino acid sequence of full-length of 1A1-Fc
QVQLVESGGGSVQAGGSLRLSCTASGYTFRGWNKHWYRQAPGKERELVSSIFRDGKTAYTDSVKGRFTISQDNADATVYLQMNSLKPEDTAMYYCKYDLPGSGLPAFWGQGTLVTVSSEPKSCDKTHTCPPCPAPELLGGPSVFLFPPKPKDTLMISRTPEVTCVVVDVSHEDPEVKFNWYVDGVEVHNAKTKPREEQYNSTYRVVSVLTVLHQDWLNGKEYKCKVSNKALPAPIEKTISKAKGQPREPQVYTLPPSRDELTKNQVSLTCLVKGFYPSDIAVEWESNGQPENNYKTTPPVLDSDGSFFLYSKLTVDKSRWQQGNVFSCSVMHEALHNHYTQKSLSLSPGK

SEQ ID NO: 28 - DNA, 1050 bp, Artificial Sequence
  the nucleotide sequence of full-length of 1A1-Fc
caagtgcaactggtggagtctggaggcggttccgtgcaggccggcggctccctgagactgtcctgcaccgcttccggctacaccttcagaggctggaacaagcactggtatcggcaggctcctggcaaagaaagagagctggtgtcctccatcttccgggacggcaagaccgcctacaccgactccgtgaagggcagattcaccatctctcaggacaacgccgacgccacagtgtacctgcagatgaactctctgaagcccgaggacaccgccatgtactactgcaagtacgacctgcctggatctggcctgcccgccttctggggccaaggcaccctggtaaccgtgtcgtccgagcccaagtcttgcgacaagacccacacctgtcctccttgtcctgctccggaactgctgggcggcccttccgtgtttctgtttcctccaaagcctaaggacacactgatgatcagccggacccctgaggtgacctgcgtggtcgtggatgtctctcacgaggatcctgaggtgaagttcaactggtacgtggatggagtggaagtgcataacgctaaaaccaagcctagagaagagcagtacaactccacctacagagtggtgtccgtgctgaccgtgctgcaccaggattggctgaacggcaaagagtacaagtgcaaggtgtccaacaaggctctgcctgcccctatcgagaagaccatctccaaggccaagggccagcctcgggagcctcaagtgtacaccctgcctccttctcgcgacgagctgaccaagaaccaggtgtctctgacctgcctggtgaaaggcttctacccctccgacatcgccgtggaatgggagtccaatggccagcccgagaacaactacaagaccaccccacctgtgctggactctgatggctccttcttcctgtactccaagctgaccgtggacaagtccagatggcagcagggcaacgtgttctcctgttctgtgatgcacgaggccctgcacaaccactacacacagaagtccctgagcctgtctcctggcaag

SEQ ID NO: 29 - protein, 355 aa, Artificial Sequence
  the amino acid sequence of full-length of 1A10-Fc
QVQLVESGGGSVQAGGSLRLSCAASGYSSNVACMAWYRQAPGKEREWVATIVADFGTTNYAASVKGRFTISQDNAKNTVYLQMNSLKPEDSAMYYCAATQRGGIDWCDEINYWGQGTLVTVSSEPKSCDKTHTCPPCPAPELLGGPSVFLFPPKPKDTLMISRTPEVTCVVVDVSHEDPEVKFNWYVDGVEVHNAKTKPREEQYNSTYRVVSVLTVLHQDWLNGKEYKCKVSNKALPAPIEKTISKAKGQPREPQVYTLPPSRDELTKNQVSLTCLVKGFYPSDIAVEWESNGQPENNYKTTPPVLDSDGSFFLYSKLTVDKSRWQQGNVFSCSVMHEALHNHYTQKSLSLSPGK

SEQ ID NO: 30 - DNA, 1065 bp, Artificial Sequence
  the nucleotide sequence of full-length of 1A10-Fc
caggtgcaactggtggagtctggcggcggatctgtgcaagctggcggatccctgagactgtcttgtgccgcttccggctactcctctaacgtggcctgtatggcctggtacagacaggcccctggcaaagaaagagagtgggtcgccaccatcgtggccgatttcggcaccaccaattacgccgcttccgtgaagggcagattcaccatctctcaggacaacgccaagaacaccgtgtacctgcagatgaactccctgaagcctgaggactccgccatgtactactgcgccgctacacagcgcggaggcattgattggtgcgacgagattaactactggggccaaggcaccctggttaccgtgtcctctgagcccaagtcctgcgacaagacccacacctgtccaccttgtcctgccccagaactgctgggcggtcccagcgtgttcctgttcccccccaagcctaaggacacactgatgatctctagaacccctgaagtgacctgcgtggtggtcgatgtatctcacgaggatcctgaggtcaagttcaactggtacgtggacggagtggaagtgcataatgctaagaccaagcctagagaggaacagtacaactccacctacagagtggtgtccgtgctgaccgtgctgcaccaggattggctgaacggcaaggagtacaagtgcaaggtgtccaacaaggctctgcctgctcctatcgagaagaccatcagcaaggccaagggccagcctcgggagcctcaagtgtacaccctgcctccttctcgggacgagctgaccaagaaccaggtgtctcttacatgcctggtgaaaggcttctacccttccgacatcgccgtggaatgggagtccaatggccagcccgagaacaactacaagaccacacctcctgtgctggactctgacggctccttcttcctgtactccaagctgacagtggataagtccagatggcagcagggcaacgtgttctcctgctccgtgatgcacgaggccctgcacaaccactacacccagaagtctctgagcctgtcccctggaaaa

SEQ ID NO: 31 - protein, 358 aa, Artificial Sequence
  the amino acid sequence of full-length of 1A11-Fc
QVQLVESGGGSVQAGGSLRLSCAASGVTFNSACMGWFRQAPGKEREGVARIETGYGGTVYADSVKGRFTISRDNAKNTVYLQMNSLKPEDTAMYYCAAKRSWCTPTWWHELDYNYWGQGTQVTVSSEPKSCDKTHTCPPCPAPELLGGPSVFLFPPKPKDTLMISRTPEVTCVVVDVSHEDPEVKFNWYVDGVEVHNAKTKPREEQYNSTYRVVSVLTVLHQDWLNGKEYKCKVSNKALPAPIEKTISKAKGQPREPQVYTLPPSRDELTKNQVSLTCLVKGFYPSDIAVEWESNGQPENNYKTTPPVLDSDGSFFLYSKLTVDKSRWQQGNVFSCSVMHEALHNHYTQKSLSLSPGK

SEQ ID NO: 32 - DNA, 1074 bp, Artificial Sequence
  the nucleotide sequence of full-length of 1A11-Fc
caggtgcagttggttgaatctggcggcggatctgtgcaggctggcggatctctgagactgtcctgtgccgcttccggcgtcaccttcaactccgcttgcatgggatggttcagacaggcccctggcaaagagagagagggcgtcgctaggatcgagaccggctatggcggaaccgtctacgccgactccgtcaagggcaggttcaccatcagcagagacaacgccaagaacaccgtgtacctgcagatgaactccctgaagcccgaggacaccgccatgtactactgtgctgccaagagaagctggtgcacccctacctggtggcacgagctggactacaactactggggccagggcacacaggtcaccgtgtcctctgagcctaagtcctgcgacaagacccacacctgtcctccatgtcctgctccagaactgctcggcggaccttccgtgttcctgtttcctccaaagcctaaggataccctgatgatctctcggacccctgaagtgacctgcgtggtggtggatgtgtctcacgaggatcccgaagtgaagttcaattggtacgtggacggcgtggaagtgcacaatgctaagaccaagcctagagaggaacagtacaactccacctatagagtggtgtccgtgctgaccgtgctgcaccaggattggctgaacggcaaagagtacaagtgcaaggtgtccaacaaggccctgcctgctcctatcgaaaagaccatctccaaggccaagggccagcctagggaaccccaggtttacaccttgcctccatctcgggacgagctgaccaagaaccaggtgtccctgacctgtctggtcaagggcttctacccctccgatatcgccgtggaatgggagtctaatggccagccagagaacaactacaagacaacccctcctgtgctggactccgacggctcattcttcctgtactccaagctgacagtggacaagtccagatggcagcagggcaacgtgttctcctgctccgtgatgcacgaggccctgcacaatcactacacccagaagtccctgtctctgagccccggcaaa

SEQ ID NO: 33 - protein, 350 aa, Artificial Sequence
  the amino acid sequence of full-length of 1B10-Fc
EVQLVESGGGSVQAGGSLRLSCTASGYTFRGWNKHWYRQAPGKERELVSSIFRDGKTAYTDSVKGRFTISQDSADATVYLQMNSLKPEDTAMYYCKYDLPGSGLPEFWGQGTLVTVSSEPKSCDKTHTCPPCPAPELLGGPSVFLFPPKPKDTLMISRTPEVTCVVVDVSHEDPEVKFNWYVDGVEVHNAKTKPREEQYNSTYRVVSVLTVLHQDWLNGKEYKCKVSNKALPAPIEKTISKAKGQPREPQVYTLPPSRDELTKNQVSLTCLVKGFYPSDIAVEWESNGQPENNYKTTPPVLDSDGSFFLYSKLTVDKSRWQQGNVFSCSVMHEALHNHYTQKSLSLSPGK

SEQ ID NO: 34 - DNA, 1050 bp, Artificial Sequence
  the nucleotide sequence of full-length of 1B10-Fc
gaggtgcaactggtggagtctggaggcggttccgtgcaggccggcggctccctgagactgtcctgcaccgcttccggctacaccttcagaggctggaacaagcactggtatcggcaggctcctggcaaagaaagagagctggtgtcctccatcttccgggacggcaagaccgcctacaccgactccgtgaagggcagattcaccatctctcaggactctgccgacgccacagtgtacctgcagatgaactctctgaagcccgaggacaccgccatgtactactgcaagtacgacctgcctggatctggcctgcccgagttctggggccaaggcaccctggtaaccgtgtcgtccgagcccaagtcttgcgacaagacccacacctgtcctccttgtcctgctccggaactgctgggcggcccttccgtgtttctgtttcctccaaagcctaaggacacactgatgatcagccggacccctgaggtgacctgcgtggtcgtggatgtctctcacgaggatcctgaggtgaagttcaactggtacgtggatggagtggaagtgcataacgctaaaaccaagcctagagaagagcagtacaactccacctacagagtggtgtccgtgctgaccgtgctgcaccaggattggctgaacggcaaagagtacaagtgcaaggtgtccaacaaggctctgcctgcccctatcgagaagaccatctccaaggccaagggccagcctcgggagcctcaagtgtacaccctgcctccttctcgcgacgagctgaccaagaaccaggtgtctctgacctgcctggtgaaaggcttctacccctccgacatcgccgtggaatgggagtccaatggccagcccgagaacaactacaagaccaccccacctgtgctggactctgatggctccttcttcctgtactccaagctgaccgtggacaagtccagatggcagcagggcaacgtgttctcctgttctgtgatgcacgaggccctgcacaaccactacacacagaagtccctgagcctgtctcctggcaag

SEQ ID NO: 35 - protein, 54 aa, Homo sapiens
MLQMAGQCSQNEYFDSLLHACIPCQLRCSSNTPPLTCQRYCNASVTNSVKGTNA

SEQ ID NO: 36 - protein, 53 aa, Macaca fascicularis
MLQMARQCSQNEYFDSLLHDCKPCQLRCSSTPPLTCQRYCNASMTNSVKGMNA